European Patent Specification EP 4 314 339 B1, published June 18, 2025. Title: Chimeric artefact detection method. Applicant: Oxford University Innovation Limited. Application EP. The sequence listing filed with the application follows.

SEQUENCE LISTING (62 sequences)

SEQ ID NO: 1 - DNA, 12 bp, synthetic construct
  source 1..12: mol_type = other DNA
aaggccttaagg

SEQ ID NO: 2 - DNA, 23 bp, synthetic construct
  source 1..23: mol_type = other DNA
aagcagtggtatcaacgcagagt

SEQ ID NO: 3 - DNA, 30 bp, synthetic construct
  source 1..30: mol_type = other DNA
  misc_feature 1..27: note = DNA
  misc_feature 28..30: note = RNA
aagcagtggtatcaacgcagagtgaatggg

SEQ ID NO: 4 - DNA, 24 bp, synthetic construct
  source 1..24: mol_type = other DNA
  misc_feature 1..21: note = DNA
  misc_feature 22..24: note = RNA
tacacgacgctcttccgatctggg

SEQ ID NO: 5 - DNA, 20 bp, synthetic construct
  source 1..20: mol_type = other DNA
gtggtatcaacgcagagtac

SEQ ID NO: 6 - DNA, 20 bp, synthetic construct
  source 1..20: mol_type = other DNA
gtccgagcgtaggttatccg

SEQ ID NO: 7 - DNA, 12 bp, synthetic construct
  source 1..12: mol_type = other DNA
aaagttgggccc

SEQ ID NO: 8 - DNA, 13 bp, synthetic construct
  source 1..13: mol_type = other DNA
aaagtttgggccc

SEQ ID NO: 9 - DNA, 12 bp, synthetic construct
  source 1..12: mol_type = other DNA
aaatttgggccc

SEQ ID NO: 10 - DNA, 65 bp, synthetic construct
  source 1..65: mol_type = other DNA
  variation 26..35: note = n is a, c, g or t
aagcagtggtatcaacgcagagtacnnnnnnnnnntttttttttttttttttttttttttttttt

SEQ ID NO: 11 - DNA, 40 bp, synthetic construct
  source 1..40: mol_type = other DNA
  variation 24..33: note = n is a, c, g or t
  misc_feature 38..40: note = RNA
  misc_feature 1..37: note = DNA
aagcagtggtatcaacgcagagtnnnnnnnnnngaatggg

SEQ ID NO: 12 - DNA, 23 bp, synthetic construct
  source 1..23: mol_type = other DNA
aagcagtggtatcaacgcagagt

SEQ ID NO: 13 - DNA, 23 bp, synthetic construct
  source 1..23: mol_type = other DNA
aagcagtggtatcaacgcagagt

SEQ ID NO: 14 - DNA, 35 bp, synthetic construct
  source 1..35: mol_type = other DNA
aaatttgggcccaagctgtggtatcaacgcagagt

SEQ ID NO: 15 - DNA, 35 bp, synthetic construct
  source 1..35: mol_type = other DNA
tttcccaaagggaagctgtggtatcaacgcagagt

SEQ ID NO: 16 - DNA, 35 bp, synthetic construct
  source 1..35: mol_type = other DNA
gggaaaccctttaagctgtggtatcaacgcagagt

SEQ ID NO: 17 - DNA, 35 bp, synthetic construct
  source 1..35: mol_type = other DNA
cccgggtttaaaaagctgtggtatcaacgcagagt

SEQ ID NO: 18 - DNA, 37 bp, synthetic construct
  source 1..37: mol_type = other DNA
gcctgtccgcggaagcagtggtatcaacgcagagtac

SEQ ID NO: 19 - DNA, 22 bp, synthetic construct
  source 1..22: mol_type = other DNA
ctacacgacgctcttccgatct

SEQ ID NO: 20 - DNA, 25 bp, synthetic construct
  source 1..25: mol_type = other DNA
gtactctgcgttgataccactgctt

SEQ ID NO: 21 - DNA, 26 bp, synthetic construct
  source 1..26: mol_type = other DNA
aagcagtggtatcaacgcagagtaat

SEQ ID NO: 22 - DNA, 30 bp, synthetic construct
  source 1..30: mol_type = other DNA
gggaaaccctttgggccctttaaacccttt

SEQ ID NO: 23 - DNA, 25 bp, synthetic construct
  source 1..25: mol_type = other DNA
gtactctgcgttgataccactgctt

SEQ ID NO: 24 - DNA, 26 bp, synthetic construct
  source 1..26: mol_type = other DNA
aagcagtggtatcaacgcagagtaat

SEQ ID NO: 25 - DNA, 15 bp, synthetic construct
  source 1..15: mol_type = other DNA
agatcggaagagcgt

SEQ ID NO: 26 - DNA, 12 bp, synthetic construct
  source 1..12: mol_type = other DNA
gtactctgcgtt

SEQ ID NO: 27 - DNA, 37 bp, synthetic construct
  source 1..37: mol_type = other DNA
tttagggcccaaagggtgtcccaaatttgggaggttt

SEQ ID NO: 28 - DNA, 12 bp, synthetic construct
  source 1..12: mol_type = other DNA
tgcagtcatggt

SEQ ID NO: 29 - DNA, 30 bp, synthetic construct
  source 1..30: mol_type = other DNA
aaatttcccgggaaagggtttggggggccc

SEQ ID NO: 30 - DNA, 33 bp, synthetic construct
  source 1..33: mol_type = other DNA
atatttcccgggaaacccgggtttggggggccc

SEQ ID NO: 31 - DNA, 30 bp, synthetic construct
  source 1..30: mol_type = other DNA
aaatttcccagggcccgggtttggggggcc

SEQ ID NO: 32 - DNA, 15 bp, synthetic construct
  source 1..15: mol_type = other DNA
aaatttcccagggaa

SEQ ID NO: 33 - DNA, 15 bp, synthetic construct
  source 1..15: mol_type = other DNA
aaatttcccgggaaa

SEQ ID NO: 34 - DNA, 12 bp, synthetic construct
  source 1..12: mol_type = other DNA
tttaaaaaaaaa

SEQ ID NO: 35 - DNA, 12 bp, synthetic construct
  source 1..12: mol_type = other DNA
gggtttaaaggg

SEQ ID NO: 36 - DNA, 12 bp, synthetic construct
  source 1..12: mol_type = other DNA
gggtttcccggg

SEQ ID NO: 37 - DNA, 12 bp, synthetic construct
  source 1..12: mol_type = other DNA
tttcccaaattt

SEQ ID NO: 38 - DNA, 12 bp, synthetic construct
  source 1..12: mol_type = other DNA
aaacccgggccc

SEQ ID NO: 39 - DNA, 12 bp, synthetic construct
  source 1..12: mol_type = other DNA
aaatttcccccc

SEQ ID NO: 40 - DNA, 12 bp, synthetic construct
  source 1..12: mol_type = other DNA
gggtttcctggg

SEQ ID NO: 41 - DNA, 12 bp, synthetic construct
  source 1..12: mol_type = other DNA
tttcccaaaatt

SEQ ID NO: 42 - DNA, 12 bp, synthetic construct
  source 1..12: mol_type = other DNA
gggcccggggga

SEQ ID NO: 43 - DNA, 12 bp, synthetic construct
  source 1..12: mol_type = other DNA
ggttttcccccc

SEQ ID NO: 44 - DNA, 10 bp, synthetic construct
  source 1..10: mol_type = other DNA
gcggactagc

SEQ ID NO: 45 - DNA, 10 bp, synthetic construct
  source 1..10: mol_type = other DNA
agtaggggtg

SEQ ID NO: 46 - DNA, 10 bp, synthetic construct
  source 1..10: mol_type = other DNA
aagtcatcta

SEQ ID NO: 47 - DNA, 10 bp, synthetic construct
  source 1..10: mol_type = other DNA
cgttcatagt

SEQ ID NO: 48 - DNA, 10 bp, synthetic construct
  source 1..10: mol_type = other DNA
aagtctgatt

SEQ ID NO: 49 - DNA, 10 bp, synthetic construct
  source 1..10: mol_type = other DNA
aagtaaccct

SEQ ID NO: 50 - DNA, 10 bp, synthetic construct
  source 1..10: mol_type = other DNA
gcgtccataa

SEQ ID NO: 51 - DNA, 10 bp, synthetic construct
  source 1..10: mol_type = other DNA
tgaaaaagac

SEQ ID NO: 52 - DNA, 10 bp, synthetic construct
  source 1..10: mol_type = other DNA
agacgtgtgt

SEQ ID NO: 53 - DNA, 10 bp, synthetic construct
  source 1..10: mol_type = other DNA
gtcagccgct

SEQ ID NO: 54 - DNA, 20 bp, synthetic construct
  source 1..20: mol_type = other DNA
aagtcatctagcatcgtcac

SEQ ID NO: 55 - DNA, 20 bp, synthetic construct
  source 1..20: mol_type = other DNA
cgttcatactaagtaaccct

SEQ ID NO: 56 - DNA, 20 bp, synthetic construct
  source 1..20: mol_type = other DNA
gcggactagctgaaaaagac

SEQ ID NO: 57 - DNA, 20 bp, synthetic construct
  source 1..20: mol_type = other DNA
aaggtcactcctcgtcggac

SEQ ID NO: 58 - DNA, 20 bp, synthetic construct
  source 1..20: mol_type = other DNA
gtcgttaagttcgattttgt

SEQ ID NO: 59 - DNA, 20 bp, synthetic construct
  source 1..20: mol_type = other DNA
aagtcatctagcatcgtcac

SEQ ID NO: 60 - DNA, 10 bp, synthetic construct
  source 1..10: mol_type = other DNA
aagtcatcta

SEQ ID NO: 61 - DNA, 20 bp, synthetic construct
  source 1..20: mol_type = other DNA
aagtcatctagcatcgtcac

SEQ ID NO: 62 - DNA, 10 bp, synthetic construct
  source 1..10: mol_type = other DNA
gcatcgtcac